European Patent Application EP 4 620 963 A1, published September 24, 2025. Title: Peptide Having Activity of Skin Whitening and Uses Thereof. Applicant: CAREGEN CO., LTD. The sequence listing filed with the application follows.

SEQUENCE LISTING (9 sequences)

SEQ ID NO: 1 - protein, 4 aa, synthetic construct
RTLE

SEQ ID NO: 2 - DNA, 20 bp, synthetic construct
  source 1..20: mol_type = other DNA
tgctagcagcctctctctcc

SEQ ID NO: 3 - DNA, 20 bp, synthetic construct
  source 1..20: mol_type = other DNA
cttcaaggggaaccagatga

SEQ ID NO: 4 - DNA, 20 bp, synthetic construct
  source 1..20: mol_type = other DNA
ggagccaaaagggtcatcat

SEQ ID NO: 5 - DNA, 20 bp, synthetic construct
  source 1..20: mol_type = other DNA
gtgatggcatggactgtggt

SEQ ID NO: 6 - DNA, 20 bp, synthetic construct
  source 1..20: mol_type = other DNA
gccgtctatttgccacacac

SEQ ID NO: 7 - DNA, 20 bp, synthetic construct
  source 1..20: mol_type = other DNA
gcagtcagcaacttcatggc

SEQ ID NO: 8 - DNA, 20 bp, synthetic construct
  source 1..20: mol_type = other DNA
tgaccaaacgtatccccctg

SEQ ID NO: 9 - DNA, 20 bp, synthetic construct
  source 1..20: mol_type = other DNA
ggtgtctgccgttgaagaga